European Patent Specification EP 3 988 118 B1, published January 28, 2026. Title: ANTI-AGING APPLICATION OF JWA GENE AND RELATED COMPOUND. Applicant: ZHOU, JIANWEI. The sequence listing filed with the application follows.

SEQUENCE LISTING (2 sequences)

SEQ ID NO: 1 - DNA, 2114 bp, Homo sapiens
gaattcggcacgagccgagacggagccgctgtcaactctccaactcagctcagctgatcggttgccgccgccgccgccgccagattctggaggcgaagaacgcaaagctgagaacatggacgttaatatcgccccactccgcgcctgggacgatttcttcccgggttccgatcgctttgcccggccggacttcagggacatttccaaatggaacaaccgcgtagtgagcaacctgctctattaccagaccaactacctggtggtggctgccatgatgatttccattgtggggtttctgagtcccttcaacatgatcctgggaggaatcgtggtggtgctggtgttcacagggtttgtgtgggcagcccacaataaagacgtccttcgccggatgaagaagcgctaccccacgacgttcgttatggtggtcatgttggcgagctatttccttatctccatgtttggaggagtcatggtctttgtgtttggcattacttttcctttgctgttgatgtttatccatgcatcgttgagacttcggaacctcaagaacaaactggagaataaaatggaaggaataggtttgaagaggacaccgatgggcattgtcctggatgccctagaacagcaggaagaaggcatcaacagactcactgactatatcagcaaagtgaaggaataaacataacttacctgagctagggttgcagcagaaattgagttgcagcttgcccttgtccagacctatgttctgcttgcgtttttgaaacaggaggtgcacgtaccacccaattatctatggcagcatgcatgtataggccgaactattatcagctctgatgtttcagagagaagacctcagaaaccgaaagaaaaccaccaccctcctattgtgtctgaagtttcacgtgtgtttatgaaatctaatgggaaatggatcacacgatttctttaagggaattaaaaaaaataaaagaattacggcttttacagcaacaatacgattatcttataggaaaaaaaaaaatcattgtaaagtatcaagacaatacgagtaaatgaaaaggctgttaaagtagatgacatcatgtgttagcctgttcctaaatccctagaattgtaatgtgtgggatataaattagtttttattattctcttaaaaatcaaagatgatctctatcactttgccacctgtttgatgtgcagtggaaactggttaagccagttgttcatacttcctttacaaatataaagatagctgtttaggatattttgttacatttttgtaaatttttgaaatgctagtaatgtgttttcaccagcaagtatttgttgcaaacttaatgtcattttccttaagatggttacagctatgtaacctgtattattctggacggacttattaaaatacaaacagacaaaaaataaaacaaaacttgagttctatttaccttgcacattttttgttgttacagtgaaaaaaatggtccaagaaaatgtttgccatttttgcattgtttcgtttttaactggaacatttagaaagaaggaaatgaatgtgcattttattaattccttaggggcacaaggaggacaataatagctgatcttttgaaatttgaaaaacgtctttagatgaccaagcaaaaagactttaaaaaatggtaatgaaaatggaatgcagctactgcagctaataaaaaattttagatagcaattgttacaaccatatgcctttatagctagacattagaattatgatagcatgagtttatacattctattatttttcctccctttctcatgtttttataaataggtaataaaaaatgttttgcctgccaattgaatgatttcgtagctgaagtagaaacatttaggtttctgtagcattaaattgtgaagacaactggagtggtacttactgaagaaactctctgtatgtcctagaataagaagcaatgatgtgctgcttctgatttttcttgcattttaaattctcagccaacctacagccatgatctttagcacagtgatatcaccatgacttcacagacatggtctagaatctgtacccttacccacatatgaagaataaaattgattaaaggtta

SEQ ID NO: 2 - protein, 188 aa, Homo sapiens
MDVNIAPLRAWDDFFPGSDRFARPDFRDISKWNNRVVSNLLYYQTNYLVVAAMMISIVGFLSPFNMILGGIVVVLVFTGFVWAAHNKDVLRRMKKRYPTTFVMVVMLASYFLISMFGGVMVFVFGITFPLLLMFIHASLRLRNLKNKLENKMEGIGLKRTPMGIVLDALEQQEEGINRLTDYISKVKE